European Patent Application EP 4 736 889 A2, published May 6, 2026. Title: COMPOSITIONS AND METHODS FOR DELIVERY OF NUCLEIC ACIDS TO CELLS. Applicant: YALE UNIVERSITY. Application EP. The sequence listing filed with the application follows.

SEQUENCE LISTING (93 sequences)

SEQ ID NO: 1 - protein, 116 aa, synthetic construct
  source 1..116: note = synthetic polypeptide
EVQLVESGGGLVKPGGSRKLSCAASGFTFSDYGMHWVRQAPEKGLEWVAYISSGSSTIYYADTVKGRFTISRDNAKNTLFLQMTSLRSEDTAMYYCARRGLLLDYWGQGTTLTVSS

SEQ ID NO: 2 - protein, 116 aa, synthetic construct
  source 1..116: note = synthetic polypeptide
EVQLVESGGGLVKPGGSRKLSCAASGFTFSNYGMHWVRQAPEKGLEWVAYISSGSSTIYYADTVKGRFTISRDNAKNTLFLQMTSLRSEDTAMYYCARRGLLLDYWGQGTTLTVSS

SEQ ID NO: 3 - protein, 116 aa, synthetic construct
  source 1..116: note = synthetic polypeptide
EVQLVQSGGGLIQPGGSLRLSCAASGFTFSNYGMHWVRQAPGKGLEWVSYISSGSSTIYYADSVKGRFTISRDNSKNTLYLQMNSLRAEDTAVYYCARRGLLLDYWGQGTTVTVSS

SEQ ID NO: 4 - protein, 116 aa, synthetic construct
  source 1..116: note = synthetic polypeptide
EVQLVESGGGLIQPGGSLRLSCAASGFTFSNYGMHWVRQAPGKGLEWVSYISSGSSTIYYADSVKGRFTISRDNSKNTLYLQMTSLRAEDTAVYYCARRGLLLDYWGQGTTLTVSS

SEQ ID NO: 5 - protein, 116 aa, synthetic construct
  source 1..116: note = synthetic polypeptide
EVQLQESGGGVVQPGGSLRLSCAASGFTFSNYGMHWIRQAPGKGLEWVSYISSGSSTIYYADSVKGRFTISRDNSKNTLYLQMNSLRSEDTAVYYCARRGLLLDYWGQGTLVTVSS

SEQ ID NO: 6 - protein, 116 aa, synthetic construct
  source 1..116: note = synthetic polypeptide
EVQLVESGGGLVQPGGSLRLSCSASGFTFSNYGMHWVRQAPGKGLEYVSYISSGSSTIYYADTVKGRFTISRDNSKNTLYLQMSSLRAEDTAVYYCVKRGLLLDYWGQGTLVTVSS

SEQ ID NO: 7 - protein, 111 aa, synthetic construct
  source 1..111: note = synthetic polypeptide
DIVLTQSPASLAVSLGQRATISCRASKSVSTSSYSYMHWYQQKPGQPPKLLIKYASYLESGVPARFSGSGSGTDFTLNIHPVEEEDAATYYCQHSREFPWTFGGGTKLEIK

SEQ ID NO: 8 - protein, 111 aa, synthetic construct
  source 1..111: note = synthetic polypeptide
DIVLTQSPASLAVSLGQRATISCRASKSVSTSSYSYMHWYQQKPGQPPKLLIKYASYLESGVPARFSGSGSGTDFHLNIHPVEEEDAATYYCQHSREFPWTFGGGTKLELK

SEQ ID NO: 9 - protein, 111 aa, synthetic construct
  source 1..111: note = synthetic polypeptide
DIQMTQSPSSLSASVGDRVTITCRASKSVSTSSYSYLAWYQQKPEKAPKLLIKYASYLQSGVPSRFSGSGSGTDFTLTISSLQPEDFATYYCQHSREFPWTFGAGTKLELK

SEQ ID NO: 10 - protein, 111 aa, synthetic construct
  source 1..111: note = synthetic polypeptide
DIQMTQSPSSLSASVGDRVTISCRASKSVSTSSYSYMHWYQQKPEKAPKLLIKYASYLQSGVPSRFSGSGSGTDFTLTISSLQPEDVATYYCQHSREFPWTFGAGTKLELK

SEQ ID NO: 11 - protein, 111 aa, synthetic construct
  source 1..111: note = synthetic polypeptide
DIVLTQSPASLAVSPGQRATITCRASKSVSTSSYSYMHWYQQKPGQPPKLLIYYASYLESGVPARFSGSGSGTDFTLTINPVEANDTANYYCQHSREFPWTFGQGTKVEIK

SEQ ID NO: 12 - protein, 465 aa, synthetic construct
  source 1..465: note = synthetic polypeptide
MGWSCIILFLVATATGVHSEVQLVESGGGLVKPGGSRKLSCAASGFTFSDYGMHWVRQAPEKGLEWVAYISSGSSTIYYADTVKGRFTISRDNAKNTLFLQMTSLRSEDTAMYYCARRGLLLDYWGQGTTLTVSAASTKGPSVFPLAPSSKSTSGGTAALGCLVKDYFPEPVTVSWNSGALTSGVHTFPAVLQSSGLYSLSSVVTVPSSSLGTQTYICNVNHKPSNTKVDKKVEPKSCDKTHTCPPCPAPELLGGPSVFLFPPKPKDTLMISRTPEVTCVVVDVSHEDPEVKFNWYVDGVEVHNAKTKPREEQYNSTYRVVSVLTVLHQDWLNGKEYKCKVSNKALPAPIEKTISKAKGQPREPQVYTLPPSRDELTKNQVSLTCLVKGFYPSDIAVEWESNGQPENNYKTTPPVLDSDGSFFLYSKLTVDKSRWQQGNVFSCSVMHEALHNHYTQKSLSLSPGK

SEQ ID NO: 13 - protein, 465 aa, synthetic construct
  source 1..465: note = synthetic polypeptide
MGWSCIILFLVATATGVHSEVQLVESGGGLVKPGGSRKLSCAASGFTFSNYGMHWVRQAPEKGLEWVAYISSGSSTIYYADTVKGRFTISRDNAKNTLFLQMTSLRSEDTAMYYCARRGLLLDYWGQGTTLTVSAASTKGPSVFPLAPSSKSTSGGTAALGCLVKDYFPEPVTVSWNSGALTSGVHTFPAVLQSSGLYSLSSVVTVPSSSLGTQTYICNVNHKPSNTKVDKKVEPKSCDKTHTCPPCPAPELLGGPSVFLFPPKPKDTLMISRTPEVTCVVVDVSHEDPEVKFNWYVDGVEVHNAKTKPREEQYNSTYRVVSVLTVLHQDWLNGKEYKCKVSNKALPAPIEKTISKAKGQPREPQVYTLPPSRDELTKNQVSLTCLVKGFYPSDIAVEWESNGQPENNYKTTPPVLDSDGSFFLYSKLTVDKSRWQQGNVFSCSVMHEALHNHYTQKSLSLSPGK

SEQ ID NO: 14 - protein, 237 aa, synthetic construct
  source 1..237: note = synthetic polypeptide
MGWSCIILFLVATATGVHSDIVLTQSPASLAVSLGQRATISCRASKSVSTSSYSYMHWYQQKPGQPPKLLIKYASYLESGVPARFSGSGSGTDFTLNIHPVEEEDAATYYCQHSREFPWTFGGGTKLEIKRTVAAPSVFIFPPSDEQLKSGTASVVCLLNNFYPREAKVQWKVDNALQSGNSQESVTEQDSKDSTYSLSSTLTLSKADYEKHKVYACEVTHQGLSSPVTKSFNRGEC

SEQ ID NO: 15 - protein, 5 aa, synthetic construct
  source 1..5: note = synthetic polypeptide
DYGMH

SEQ ID NO: 16 - protein, 5 aa, synthetic construct
  source 1..5: note = synthetic polypeptide
NYGMH

SEQ ID NO: 17 - protein, 17 aa, synthetic construct
  source 1..17: note = synthetic polypeptide
YISSGSSTIYYADTVKG

SEQ ID NO: 18 - protein, 7 aa, synthetic construct
  source 1..7: note = synthetic polypeptide
RGLLLDY

SEQ ID NO: 19 - protein, 17 aa, synthetic construct
  source 1..17: note = synthetic polypeptide
YISSGSSTIYYADSVKG

SEQ ID NO: 20 - protein, 8 aa, synthetic construct
  source 1..8: note = synthetic polypeptide
GFTFSDYG

SEQ ID NO: 21 - protein, 8 aa, synthetic construct
  source 1..8: note = synthetic polypeptide
GFTFSNYG

SEQ ID NO: 22 - protein, 8 aa, synthetic construct
  source 1..8: note = synthetic polypeptide
ISSGSSTI

SEQ ID NO: 23 - protein, 9 aa, synthetic construct
  source 1..9: note = synthetic polypeptide
ARRGLLLDY

SEQ ID NO: 24 - protein, 15 aa, synthetic construct
  source 1..15: note = synthetic polypeptide
RASKSVSTSSYSYMH

SEQ ID NO: 25 - protein, 7 aa, synthetic construct
  source 1..7: note = synthetic polypeptide
YASYLES

SEQ ID NO: 26 - protein, 9 aa, synthetic construct
  source 1..9: note = synthetic polypeptide
QHSREFPWT

SEQ ID NO: 27 - protein, 15 aa, synthetic construct
  source 1..15: note = synthetic polypeptide
RASKSVSTSSYSYLA

SEQ ID NO: 28 - protein, 7 aa, synthetic construct
  source 1..7: note = synthetic polypeptide
YASYLQS

SEQ ID NO: 29 - protein, 10 aa, synthetic construct
  source 1..10: note = synthetic polypeptide
KSVSTSSYSY

SEQ ID NO: 30 - skipped

SEQ ID NO: 31 - protein, 7 aa, synthetic construct
  source 1..7: note = synthetic polypeptide
GQSSRSS

SEQ ID NO: 32 - protein, 18 aa, synthetic construct
  source 1..18: note = synthetic polypeptide
GQSSRSSSGGGSSGGGGS

SEQ ID NO: 33 - protein, 4 aa, synthetic construct
  source 1..4: note = synthetic polypeptide
GSGS

SEQ ID NO: 34 - protein, 4 aa, synthetic construct
  source 1..4: note = synthetic polypeptide
GGGS

SEQ ID NO: 35 - protein, 10 aa, synthetic construct
  source 1..10: note = synthetic polypeptide
GGGGSGGGGS

SEQ ID NO: 36 - protein, 20 aa, synthetic construct
  source 1..20: note = synthetic polypeptide
GGGGSGGGGSGGGGSGGGGS

SEQ ID NO: 37 - protein, 15 aa, synthetic construct
  source 1..15: note = synthetic polypeptide
GGGGSGGGGSGGGGS

SEQ ID NO: 38 - protein, 274 aa, synthetic construct
  source 1..274: note = synthetic polypeptide
AGIHDIVLTQSPASLAVSLGQRATISCRASKSVSTSSYSYMHWYQQKPGQPPKLLIKYASYLESGVPARFSGSGSGTDFTLNIHPVEEEDAATYYCQHSREFPWTFGGGTKLEIKRADAAPGGGGSGGGGSGGGGSEVQLVESGGGLVKPGGSRKLSCAASGFTFSNYGMHWVRQAPEKGLEWVAYISSGSSTIYYADTVKGRFTISRDNAKNTLFLQMTSLRSEDTAMYYCARRGLLLDYWGQGTTLTVSSLEQKLISEEDLNSAVDHHHHHH

SEQ ID NO: 39 - protein, 541 aa, synthetic construct
  source 1..541: note = synthetic polypeptide
AGIHDIVLTQSPASLAVSLGQRATISCRASKSVSTSSYSYMHWYQQKPGQPPKLLIKYASYLESGVPARFSGSGSGTDFTLNIHPVEEEDAATYYCQHSREFPWTFGGGTKLEIKRADAAPGGGGSGGGGSGGGGSEVQLVESGGGLVKPGGSRKLSCAASGFTFSNYGMHWVRQAPEKGLEWVAYISSGSSTIYYADTVKGRFTISRDNAKNTLFLQMTSLRSEDTAMYYCARRGLLLDYWGQGTTLTVSSASTKGPSVFPLAPLESSGSDIVLTQSPASLAVSLGQRATISCRASKSVSTSSYSYMHWYQQKPGQPPKLLIKYASYLESGVPARFSGSGSGTDFTLNIHPVEEEDAATYYCQHSREFPWTFGGGTKLEIKRADAAPGGGGSGGGGSGGGGSEVQLVESGGGLVKPGGSRKLSCAASGFTFSNYGMHWVRQAPEKGLEWVAYISSGSSTIYYADTVKGRFTISRDNAKNTLFLQMTSLRSEDTAMYYCARRGLLLDYWGQGTTLTVSSLEQKLISEEDLNSAVDHHHHHH

SEQ ID NO: 40 - protein, 808 aa, synthetic construct
  source 1..808: note = synthetic polypeptide
AGIHDIVLTQSPASLAVSLGQRATISCRASKSVSTSSYSYMHWYQQKPGQPPKLLIKYASYLESGVPARFSGSGSGTDFTLNIHPVEEEDAATYYCQHSREFPWTFGGGTKLEIKRADAAPGGGGSGGGGSGGGGSEVQLVESGGGLVKPGGSRKLSCAASGFTFSNYGMHWVRQAPEKGLEWVAYISSGSSTIYYADTVKGRFTISRDNAKNTLFLQMTSLRSEDTAMYYCARRGLLLDYWGQGTTLTVSSASTKGPSVFPLAPLESSGSDIVLTQSPASLAVSLGQRATISCRASKSVSTSSYSYMHWYQQKPGQPPKLLIKYASYLESGVPARFSGSGSGTDFTLNIHPVEEEDAATYYCQHSREFPWTFGGGTKLEIKRADAAPGGGGSGGGGSGGGGSEVQLVESGGGLVKPGGSRKLSCAASGFTFSNYGMHWVRQAPEKGLEWVAYISSGSSTIYYADTVKGRFTISRDNAKNTLFLQMTSLRSEDTAMYYCARRGLLLDYWGQGTTLTVSSASTKGPSVFPLAPLESSGSDIVLTQSPASLAVSLGQRATISCRASKSVSTSSYSYMHWYQQKPGQPPKLLIKYASYLESGVPARFSGSGSGTDFTLNIHPVEEEDAATYYCQHSREFPWTFGGGTKLEIKRADAAPGGGGSGGGGSGGGGSEVQLVESGGGLVKPGGSRKLSCAASGFTFSNYGMHWVRQAPEKGLEWVAYISSGSSTIYYADTVKGRFTISRDNAKNTLFLQMTSLRSEDTAMYYCARRGLLLDYWGQGTTLTVSSLEQKLISEEDLNSAVDHHHHHH

SEQ ID NO: 41 - protein, 242 aa, synthetic construct
  source 1..242: note = synthetic polypeptide
DIVLTQSPASLAVSPGQRATITCRASKSVSTSSYSYMHWYQQKPGQPPKLLIYYASYLESGVPARFSGSGSGTDFTLTINPVEANDTANYYCQHSREFPWTFGQGTKVEIKGGGGSGGGGSGGGGSEVQLVESGGGLVQPGGSLRLSCSASGFTFSNYGMHWVRQAPGKGLEYVSYISSGSSTIYYADTVKGRFTISRDNSKNTLYLQMSSLRAEDTAVYYCVKRGLLLDYWGQGTLVTVSS

SEQ ID NO: 42 - protein, 17 aa, synthetic construct
  source 1..17: note = synthetic polypeptide
YISSSSSTIYYADSVKG

SEQ ID NO: 43 - protein, 8 aa, synthetic construct
  source 1..8: note = synthetic polypeptide
ISSSSSTI

SEQ ID NO: 44 - protein, 15 aa, synthetic construct
  source 1..15: note = synthetic polypeptide
RASKTVSTSSYSYMH

SEQ ID NO: 45 - protein, 10 aa, synthetic construct
  source 1..10: note = synthetic polypeptide
KTVSTSSYSY

SEQ ID NO: 46 - protein, 116 aa, synthetic construct
  source 1..116: note = synthetic polypeptide
EVQLVESGGGLVQPGGSLRLSCAASGFTFSNYGMHWVRQAPGKGLEWVSYISSSSSTIYYADSVKGRFTISRDNAKNSLYLQMNSLRAEDTAVYYCARRGLLLDYWGQGTTVTVSS

SEQ ID NO: 47 - protein, 116 aa, synthetic construct
  source 1..116: note = synthetic polypeptide
EVQLVESGGGVVQPGGSLRLSCAASGFTFSNYGMHWVRQAPEKGLEWVSYISSSSSTIYYADSVKGRFTISRDNSKNTLYLQMNSLRAEDTAVYYCARRGLLLDYWGQGTTVTVSS

SEQ ID NO: 48 - protein, 116 aa, synthetic construct
  source 1..116: note = synthetic polypeptide
EVQLVESGGGDVKPGGSLRLSCAASGFTFSNYGMHWVRQAPEKGLEWVSYISSSSSTIYYADSVKGRFTISRDNSKNTLYLQMNSLRAEDTAVYYCARRGLLLDYWGQGTTVTVSS

SEQ ID NO: 49 - skipped

SEQ ID NO: 50 - protein, 116 aa, synthetic construct
  source 1..116: note = synthetic polypeptide
EVQLVESGGGLVQPGGSLRLSCAASGFTFSNYGMHWVRQAPGKGLEWVSYISSGSSTIYYADSVKGRFTISRDNAKNSLYLQMNSLRAEDTAVYYCARRGLLLDYWGQGTTVTVSS

SEQ ID NO: 51 - protein, 116 aa, synthetic construct
  source 1..116: note = synthetic polypeptide
EVQLVESGGGVVQPGGSLRLSCAASGFTFSNYGMHWVRQAPEKGLEWVSYISSGSSTIYYADSVKGRFTISRDNSKNTLYLQMNSLRAEDTAVYYCARRGLLLDYWGQGTTVTVSS

SEQ ID NO: 52 - protein, 116 aa, synthetic construct
  source 1..116: note = synthetic polypeptide
EVQLVESGGGDVKPGGSLRLSCAASGFTFSNYGMHWVRQAPEKGLEWVSYISSGSSTIYYADSVKGRFTISRDNSKNTLYLQMNSLRAEDTAVYYCARRGLLLDYWGQGTTVTVSS

SEQ ID NO: 53 - protein, 111 aa, synthetic construct
  source 1..111: note = synthetic polypeptide
DIQMTQSPSSLSASLGDRATITCRASKSVSTSSYSYMHWYQQKPGQPPKLLIKYASYLESGVPSRFSGSGSGTDFTLTISSLQPEDAATYYCQHSREFPWTFGGGTKVEIK

SEQ ID NO: 54 - protein, 111 aa, synthetic construct
  source 1..111: note = synthetic polypeptide
DIQMTQSPSSLSASLGDRATITCRASKSVSTSSYSYMHWYQQKPGQAPKLLIKYASYLESGVPSRFSGSGSGTDFTLTISSLQPEDFATYYCQHSREFPWTFGQGTKVEIK

SEQ ID NO: 55 - protein, 111 aa, synthetic construct
  source 1..111: note = synthetic polypeptide
DIQMTQSPSSLSASVGDRVTITCRASKSVSTSSYSYMHWYQQKPGKAPKLLIKYASYLESGVPSRFSGSGSGTDFTLTISSLQPEDFATYYCQHSREFPWTFGQGTKVEIK

SEQ ID NO: 56 - protein, 111 aa, synthetic construct
  source 1..111: note = synthetic polypeptide
DIQMTQSPSSLSASLGDRATITCRASKTVSTSSYSYMHWYQQKPGQPPKLLIKYASYLESGVPSRFSGSGSGTDFTLTISSLQPEDAATYYCQHSREFPWTFGGGTKVEIK

SEQ ID NO: 57 - protein, 111 aa, synthetic construct
  source 1..111: note = synthetic polypeptide
DIQMTQSPSSLSASVGDRVTITCRASKTVSTSSYSYMHWYQQKPGKAPKLLIKYASYLESGVPSRFSGSGSGTDFTLTISSLQPEDFATYYCQHSREFPWTFGQGTKVEIK

SEQ ID NO: 58 - protein, 111 aa, synthetic construct
  source 1..111: note = synthetic polypeptide
DIQMTQSPSSLSASLGDRATITCRASKTVSTSSYSYMHWYQQKPGQAPKLLIKYASYLESGVPSRFSGSGSGTDFTLTISSLQPEDFATYYCQHSREFPWTFGQGTKVEIK

SEQ ID NO: 59 - protein, 21 aa, synthetic construct
  source 1..21: note = synthetic polypeptide
RADAAPGGGGSGGGGSGGGGS

SEQ ID NO: 60 - protein, 19 aa, synthetic construct
  source 1..19: note = synthetic polypeptide
ASTKGPSVFPLAPLESSGS

SEQ ID NO: 61 - protein, 515 aa, synthetic construct
  source 1..515: note = synthetic polypeptide
DIQMTQSPSSLSASLGDRATITCRASKSVSTSSYSYMHWYQQKPGQPPKLLIKYASYLESGVPSRFSGSGSGTDFTLTISSLQPEDAATYYCQHSREFPWTFGGGTKVEIKRADAAPGGGGSGGGGSGGGGSEVQLVESGGGLVQPGGSLRLSCAASGFTFSNYGMHWVRQAPGKGLEWVSYISSSSSTIYYADSVKGRFTISRDNAKNSLYLQMNSLRAEDTAVYYCARRGLLLDYWGQGTTVTVSSASTKGPSVFPLAPLESSGSDIQMTQSPSSLSASLGDRATITCRASKSVSTSSYSYMHWYQQKPGQPPKLLIKYASYLESGVPSRFSGSGSGTDFTLTISSLQPEDAATYYCQHSREFPWTFGGGTKVEIKRADAAPGGGGSGGGGSGGGGSEVQLVESGGGLVQPGGSLRLSCAASGFTFSNYGMHWVRQAPGKGLEWVSYISSSSSTIYYADSVKGRFTISRDNAKNSLYLQMNSLRAEDTAVYYCARRGLLLDYWGQGTTVTVSS

SEQ ID NO: 62 - protein, 515 aa, synthetic construct
  source 1..515: note = synthetic polypeptide
DIQMTQSPSSLSASLGDRATITCRASKSVSTSSYSYMHWYQQKPGQPPKLLIKYASYLESGVPSRFSGSGSGTDFTLTISSLQPEDAATYYCQHSREFPWTFGGGTKVEIKRADAAPGGGGSGGGGSGGGGSEVQLVESGGGVVQPGGSLRLSCAASGFTFSNYGMHWVRQAPEKGLEWVSYISSSSSTIYYADSVKGRFTISRDNSKNTLYLQMNSLRAEDTAVYYCARRGLLLDYWGQGTTVTVSSASTKGPSVFPLAPLESSGSDIQMTQSPSSLSASLGDRATITCRASKSVSTSSYSYMHWYQQKPGQPPKLLIKYASYLESGVPSRFSGSGSGTDFTLTISSLQPEDAATYYCQHSREFPWTFGGGTKVEIKRADAAPGGGGSGGGGSGGGGSEVQLVESGGGVVQPGGSLRLSCAASGFTFSNYGMHWVRQAPEKGLEWVSYISSSSSTIYYADSVKGRFTISRDNSKNTLYLQMNSLRAEDTAVYYCARRGLLLDYWGQGTTVTVSS

SEQ ID NO: 63 - protein, 515 aa, synthetic construct
  source 1..515: note = synthetic polypeptide
DIQMTQSPSSLSASLGDRATITCRASKSVSTSSYSYMHWYQQKPGQPPKLLIKYASYLESGVPSRFSGSGSGTDFTLTISSLQPEDAATYYCQHSREFPWTFGGGTKVEIKRADAAPGGGGSGGGGSGGGGSEVQLVESGGGDVKPGGSLRLSCAASGFTFSNYGMHWVRQAPEKGLEWVSYISSSSSTIYYADSVKGRFTISRDNSKNTLYLQMNSLRAEDTAVYYCARRGLLLDYWGQGTTVTVSSASTKGPSVFPLAPLESSGSDIQMTQSPSSLSASLGDRATITCRASKSVSTSSYSYMHWYQQKPGQPPKLLIKYASYLESGVPSRFSGSGSGTDFTLTISSLQPEDAATYYCQHSREFPWTFGGGTKVEIKRADAAPGGGGSGGGGSGGGGSEVQLVESGGGDVKPGGSLRLSCAASGFTFSNYGMHWVRQAPEKGLEWVSYISSSSSTIYYADSVKGRFTISRDNSKNTLYLQMNSLRAEDTAVYYCARRGLLLDYWGQGTTVTVSS

SEQ ID NO: 64 - protein, 515 aa, synthetic construct
  source 1..515: note = synthetic polypeptide
DIQMTQSPSSLSASLGDRATITCRASKSVSTSSYSYMHWYQQKPGQAPKLLIKYASYLESGVPSRFSGSGSGTDFTLTISSLQPEDFATYYCQHSREFPWTFGQGTKVEIKRADAAPGGGGSGGGGSGGGGSEVQLVESGGGLVQPGGSLRLSCAASGFTFSNYGMHWVRQAPGKGLEWVSYISSSSSTIYYADSVKGRFTISRDNAKNSLYLQMNSLRAEDTAVYYCARRGLLLDYWGQGTTVTVSSASTKGPSVFPLAPLESSGSDIQMTQSPSSLSASLGDRATITCRASKSVSTSSYSYMHWYQQKPGQAPKLLIKYASYLESGVPSRFSGSGSGTDFTLTISSLQPEDFATYYCQHSREFPWTFGQGTKVEIKRADAAPGGGGSGGGGSGGGGSEVQLVESGGGLVQPGGSLRLSCAASGFTFSNYGMHWVRQAPGKGLEWVSYISSSSSTIYYADSVKGRFTISRDNAKNSLYLQMNSLRAEDTAVYYCARRGLLLDYWGQGTTVTVSS

SEQ ID NO: 65 - protein, 515 aa, synthetic construct
  source 1..515: note = synthetic polypeptide
DIQMTQSPSSLSASLGDRATITCRASKSVSTSSYSYMHWYQQKPGQAPKLLIKYASYLESGVPSRFSGSGSGTDFTLTISSLQPEDFATYYCQHSREFPWTFGQGTKVEIKRADAAPGGGGSGGGGSGGGGSEVQLVESGGGVVQPGGSLRLSCAASGFTFSNYGMHWVRQAPEKGLEWVSYISSSSSTIYYADSVKGRFTISRDNSKNTLYLQMNSLRAEDTAVYYCARRGLLLDYWGQGTTVTVSSASTKGPSVFPLAPLESSGSDIQMTQSPSSLSASLGDRATITCRASKSVSTSSYSYMHWYQQKPGQAPKLLIKYASYLESGVPSRFSGSGSGTDFTLTISSLQPEDFATYYCQHSREFPWTFGQGTKVEIKRADAAPGGGGSGGGGSGGGGSEVQLVESGGGVVQPGGSLRLSCAASGFTFSNYGMHWVRQAPEKGLEWVSYISSSSSTIYYADSVKGRFTISRDNSKNTLYLQMNSLRAEDTAVYYCARRGLLLDYWGQGTTVTVSS

SEQ ID NO: 66 - protein, 515 aa, synthetic construct
  source 1..515: note = synthetic polypeptide
DIQMTQSPSSLSASLGDRATITCRASKSVSTSSYSYMHWYQQKPGQAPKLLIKYASYLESGVPSRFSGSGSGTDFTLTISSLQPEDFATYYCQHSREFPWTFGQGTKVEIKRADAAPGGGGSGGGGSGGGGSEVQLVESGGGDVKPGGSLRLSCAASGFTFSNYGMHWVRQAPEKGLEWVSYISSSSSTIYYADSVKGRFTISRDNSKNTLYLQMNSLRAEDTAVYYCARRGLLLDYWGQGTTVTVSSASTKGPSVFPLAPLESSGSDIQMTQSPSSLSASLGDRATITCRASKSVSTSSYSYMHWYQQKPGQAPKLLIKYASYLESGVPSRFSGSGSGTDFTLTISSLQPEDFATYYCQHSREFPWTFGQGTKVEIKRADAAPGGGGSGGGGSGGGGSEVQLVESGGGDVKPGGSLRLSCAASGFTFSNYGMHWVRQAPEKGLEWVSYISSSSSTIYYADSVKGRFTISRDNSKNTLYLQMNSLRAEDTAVYYCARRGLLLDYWGQGTTVTVSS

SEQ ID NO: 67 - protein, 515 aa, synthetic construct
  source 1..515: note = synthetic polypeptide
DIQMTQSPSSLSASVGDRVTITCRASKSVSTSSYSYMHWYQQKPGKAPKLLIKYASYLESGVPSRFSGSGSGTDFTLTISSLQPEDFATYYCQHSREFPWTFGQGTKVEIKRADAAPGGGGSGGGGSGGGGSEVQLVESGGGLVQPGGSLRLSCAASGFTFSNYGMHWVRQAPGKGLEWVSYISSSSSTIYYADSVKGRFTISRDNAKNSLYLQMNSLRAEDTAVYYCARRGLLLDYWGQGTTVTVSSASTKGPSVFPLAPLESSGSDIQMTQSPSSLSASVGDRVTITCRASKSVSTSSYSYMHWYQQKPGKAPKLLIKYASYLESGVPSRFSGSGSGTDFTLTISSLQPEDFATYYCQHSREFPWTFGQGTKVEIKRADAAPGGGGSGGGGSGGGGSEVQLVESGGGLVQPGGSLRLSCAASGFTFSNYGMHWVRQAPGKGLEWVSYISSSSSTIYYADSVKGRFTISRDNAKNSLYLQMNSLRAEDTAVYYCARRGLLLDYWGQGTTVTVSS

SEQ ID NO: 68 - protein, 515 aa, synthetic construct
  source 1..515: note = synthetic polypeptide
DIQMTQSPSSLSASVGDRVTITCRASKSVSTSSYSYMHWYQQKPGKAPKLLIKYASYLESGVPSRFSGSGSGTDFTLTISSLQPEDFATYYCQHSREFPWTFGQGTKVEIKRADAAPGGGGSGGGGSGGGGSEVQLVESGGGVVQPGGSLRLSCAASGFTFSNYGMHWVRQAPEKGLEWVSYISSSSSTIYYADSVKGRFTISRDNSKNTLYLQMNSLRAEDTAVYYCARRGLLLDYWGQGTTVTVSSASTKGPSVFPLAPLESSGSDIQMTQSPSSLSASVGDRVTITCRASKSVSTSSYSYMHWYQQKPGKAPKLLIKYASYLESGVPSRFSGSGSGTDFTLTISSLQPEDFATYYCQHSREFPWTFGQGTKVEIKRADAAPGGGGSGGGGSGGGGSEVQLVESGGGVVQPGGSLRLSCAASGFTFSNYGMHWVRQAPEKGLEWVSYISSSSSTIYYADSVKGRFTISRDNSKNTLYLQMNSLRAEDTAVYYCARRGLLLDYWGQGTTVTVSS

SEQ ID NO: 69 - protein, 515 aa, synthetic construct
  source 1..515: note = synthetic polypeptide
DIQMTQSPSSLSASVGDRVTITCRASKSVSTSSYSYMHWYQQKPGKAPKLLIKYASYLESGVPSRFSGSGSGTDFTLTISSLQPEDFATYYCQHSREFPWTFGQGTKVEIKRADAAPGGGGSGGGGSGGGGSEVQLVESGGGDVKPGGSLRLSCAASGFTFSNYGMHWVRQAPEKGLEWVSYISSSSSTIYYADSVKGRFTISRDNSKNTLYLQMNSLRAEDTAVYYCARRGLLLDYWGQGTTVTVSSASTKGPSVFPLAPLESSGSDIQMTQSPSSLSASVGDRVTITCRASKSVSTSSYSYMHWYQQKPGKAPKLLIKYASYLESGVPSRFSGSGSGTDFTLTISSLQPEDFATYYCQHSREFPWTFGQGTKVEIKRADAAPGGGGSGGGGSGGGGSEVQLVESGGGDVKPGGSLRLSCAASGFTFSNYGMHWVRQAPEKGLEWVSYISSSSSTIYYADSVKGRFTISRDNSKNTLYLQMNSLRAEDTAVYYCARRGLLLDYWGQGTTVTVSS

SEQ ID NO: 70 - protein, 515 aa, synthetic construct
  source 1..515: note = synthetic polypeptide
DIQMTQSPSSLSASLGDRATITCRASKTVSTSSYSYMHWYQQKPGQPPKLLIKYASYLESGVPSRFSGSGSGTDFTLTISSLQPEDAATYYCQHSREFPWTFGGGTKVEIKRADAAPGGGGSGGGGSGGGGSEVQLVESGGGLVQPGGSLRLSCAASGFTFSNYGMHWVRQAPGKGLEWVSYISSGSSTIYYADSVKGRFTISRDNAKNSLYLQMNSLRAEDTAVYYCARRGLLLDYWGQGTTVTVSSASTKGPSVFPLAPLESSGSDIQMTQSPSSLSASLGDRATITCRASKTVSTSSYSYMHWYQQKPGQPPKLLIKYASYLESGVPSRFSGSGSGTDFTLTISSLQPEDAATYYCQHSREFPWTFGGGTKVEIKRADAAPGGGGSGGGGSGGGGSEVQLVESGGGLVQPGGSLRLSCAASGFTFSNYGMHWVRQAPGKGLEWVSYISSGSSTIYYADSVKGRFTISRDNAKNSLYLQMNSLRAEDTAVYYCARRGLLLDYWGQGTTVTVSS

SEQ ID NO: 71 - protein, 515 aa, synthetic construct
  source 1..515: note = synthetic polypeptide
DIQMTQSPSSLSASLGDRATITCRASKTVSTSSYSYMHWYQQKPGQPPKLLIKYASYLESGVPSRFSGSGSGTDFTLTISSLQPEDAATYYCQHSREFPWTFGGGTKVEIKRADAAPGGGGSGGGGSGGGGSEVQLVESGGGVVQPGGSLRLSCAASGFTFSNYGMHWVRQAPEKGLEWVSYISSGSSTIYYADSVKGRFTISRDNSKNTLYLQMNSLRAEDTAVYYCARRGLLLDYWGQGTTVTVSSASTKGPSVFPLAPLESSGSDIQMTQSPSSLSASLGDRATITCRASKTVSTSSYSYMHWYQQKPGQPPKLLIKYASYLESGVPSRFSGSGSGTDFTLTISSLQPEDAATYYCQHSREFPWTFGGGTKVEIKRADAAPGGGGSGGGGSGGGGSEVQLVESGGGVVQPGGSLRLSCAASGFTFSNYGMHWVRQAPEKGLEWVSYISSGSSTIYYADSVKGRFTISRDNSKNTLYLQMNSLRAEDTAVYYCARRGLLLDYWGQGTTVTVSS

SEQ ID NO: 72 - protein, 515 aa, synthetic construct
  source 1..515: note = synthetic polypeptide
DIQMTQSPSSLSASLGDRATITCRASKTVSTSSYSYMHWYQQKPGQPPKLLIKYASYLESGVPSRFSGSGSGTDFTLTISSLQPEDAATYYCQHSREFPWTFGGGTKVEIKRADAAPGGGGSGGGGSGGGGSEVQLVESGGGDVKPGGSLRLSCAASGFTFSNYGMHWVRQAPEKGLEWVSYISSGSSTIYYADSVKGRFTISRDNSKNTLYLQMNSLRAEDTAVYYCARRGLLLDYWGQGTTVTVSSASTKGPSVFPLAPLESSGSDIQMTQSPSSLSASLGDRATITCRASKTVSTSSYSYMHWYQQKPGQPPKLLIKYASYLESGVPSRFSGSGSGTDFTLTISSLQPEDAATYYCQHSREFPWTFGGGTKVEIKRADAAPGGGGSGGGGSGGGGSEVQLVESGGGDVKPGGSLRLSCAASGFTFSNYGMHWVRQAPEKGLEWVSYISSGSSTIYYADSVKGRFTISRDNSKNTLYLQMNSLRAEDTAVYYCARRGLLLDYWGQGTTVTVSS

SEQ ID NO: 73 - protein, 515 aa, synthetic construct
  source 1..515: note = synthetic polypeptide
DIQMTQSPSSLSASVGDRVTITCRASKTVSTSSYSYMHWYQQKPGKAPKLLIKYASYLESGVPSRFSGSGSGTDFTLTISSLQPEDFATYYCQHSREFPWTFGQGTKVEIKRADAAPGGGGSGGGGSGGGGSEVQLVESGGGLVQPGGSLRLSCAASGFTFSNYGMHWVRQAPGKGLEWVSYISSGSSTIYYADSVKGRFTISRDNAKNSLYLQMNSLRAEDTAVYYCARRGLLLDYWGQGTTVTVSSASTKGPSVFPLAPLESSGSDIQMTQSPSSLSASVGDRVTITCRASKTVSTSSYSYMHWYQQKPGKAPKLLIKYASYLESGVPSRFSGSGSGTDFTLTISSLQPEDFATYYCQHSREFPWTFGQGTKVEIKRADAAPGGGGSGGGGSGGGGSEVQLVESGGGLVQPGGSLRLSCAASGFTFSNYGMHWVRQAPGKGLEWVSYISSGSSTIYYADSVKGRFTISRDNAKNSLYLQMNSLRAEDTAVYYCARRGLLLDYWGQGTTVTVSS

SEQ ID NO: 74 - protein, 515 aa, synthetic construct
  source 1..515: note = synthetic polypeptide
DIQMTQSPSSLSASVGDRVTITCRASKTVSTSSYSYMHWYQQKPGKAPKLLIKYASYLESGVPSRFSGSGSGTDFTLTISSLQPEDFATYYCQHSREFPWTFGQGTKVEIKRADAAPGGGGSGGGGSGGGGSEVQLVESGGGVVQPGGSLRLSCAASGFTFSNYGMHWVRQAPEKGLEWVSYISSGSSTIYYADSVKGRFTISRDNSKNTLYLQMNSLRAEDTAVYYCARRGLLLDYWGQGTTVTVSSASTKGPSVFPLAPLESSGSDIQMTQSPSSLSASVGDRVTITCRASKTVSTSSYSYMHWYQQKPGKAPKLLIKYASYLESGVPSRFSGSGSGTDFTLTISSLQPEDFATYYCQHSREFPWTFGQGTKVEIKRADAAPGGGGSGGGGSGGGGSEVQLVESGGGVVQPGGSLRLSCAASGFTFSNYGMHWVRQAPEKGLEWVSYISSGSSTIYYADSVKGRFTISRDNSKNTLYLQMNSLRAEDTAVYYCARRGLLLDYWGQGTTVTVSS

SEQ ID NO: 75 - protein, 515 aa, synthetic construct
  source 1..515: note = synthetic polypeptide
DIQMTQSPSSLSASVGDRVTITCRASKTVSTSSYSYMHWYQQKPGKAPKLLIKYASYLESGVPSRFSGSGSGTDFTLTISSLQPEDFATYYCQHSREFPWTFGQGTKVEIKRADAAPGGGGSGGGGSGGGGSEVQLVESGGGDVKPGGSLRLSCAASGFTFSNYGMHWVRQAPEKGLEWVSYISSGSSTIYYADSVKGRFTISRDNSKNTLYLQMNSLRAEDTAVYYCARRGLLLDYWGQGTTVTVSSASTKGPSVFPLAPLESSGSDIQMTQSPSSLSASVGDRVTITCRASKTVSTSSYSYMHWYQQKPGKAPKLLIKYASYLESGVPSRFSGSGSGTDFTLTISSLQPEDFATYYCQHSREFPWTFGQGTKVEIKRADAAPGGGGSGGGGSGGGGSEVQLVESGGGDVKPGGSLRLSCAASGFTFSNYGMHWVRQAPEKGLEWVSYISSGSSTIYYADSVKGRFTISRDNSKNTLYLQMNSLRAEDTAVYYCARRGLLLDYWGQGTTVTVSS

SEQ ID NO: 76 - protein, 515 aa, synthetic construct
  source 1..515: note = synthetic polypeptide
DIQMTQSPSSLSASLGDRATITCRASKTVSTSSYSYMHWYQQKPGQAPKLLIKYASYLESGVPSRFSGSGSGTDFTLTISSLQPEDFATYYCQHSREFPWTFGQGTKVEIKRADAAPGGGGSGGGGSGGGGSEVQLVESGGGLVQPGGSLRLSCAASGFTFSNYGMHWVRQAPGKGLEWVSYISSGSSTIYYADSVKGRFTISRDNAKNSLYLQMNSLRAEDTAVYYCARRGLLLDYWGQGTTVTVSSASTKGPSVFPLAPLESSGSDIQMTQSPSSLSASLGDRATITCRASKTVSTSSYSYMHWYQQKPGQAPKLLIKYASYLESGVPSRFSGSGSGTDFTLTISSLQPEDFATYYCQHSREFPWTFGQGTKVEIKRADAAPGGGGSGGGGSGGGGSEVQLVESGGGLVQPGGSLRLSCAASGFTFSNYGMHWVRQAPGKGLEWVSYISSGSSTIYYADSVKGRFTISRDNAKNSLYLQMNSLRAEDTAVYYCARRGLLLDYWGQGTTVTVSS

SEQ ID NO: 77 - protein, 446 aa, synthetic construct
  source 1..446: note = synthetic polypeptide
EVQLVESGGGLVQPGGSLRLSCAASGFTFSNYGMHWVRQAPGKGLEWVSYISSGSSTIYYADSVKGRFTISRDNAKNSLYLQMNSLRAEDTAVYYCARRGLLLDYWGQGTTVTVSSASTKGPSVFPLAPSSKSTSGGTAALGCLVKDYFPEPVTVSWNSGALTSGVHTFPAVLQSSGLYSLSSVVTVPSSSLGTQTYICNVNHKPSNTKVDKKVEPKSCDKTHTCPPCPAPEAAGGPSVFLFPPKPKDTLMISRTPEVTCVVVDVSHEDPEVKFNWYVDGVEVHNAKTKPREEQYNSTYRVVSVLTVLHQDWLNGKEYKCKVSNKALPAPIEKTISKAKGQPREPQVYTLPPSRDELTKNQVSLTCLVKGFYPSDIAVEWESNGQPENNYKTTPPVLDSDGSFFLYSKLTVDKSRWQQGNVFSCSVMHEALHNHYTQKSLSLSPGK

SEQ ID NO: 78 - protein, 98 aa, synthetic construct
  source 1..98: note = synthetic polypeptide
ASTKGPSVFPLAPSSKSTSGGTAALGCLVKDYFPEPVTVSWNSGALTSGVHTFPAVLQSSGLYSLSSVVTVPSSSLGTQTYICNVNHKPSNTKVDKKV

SEQ ID NO: 79 - protein, 12 aa, synthetic construct
  source 1..12: note = synthetic polypeptide
EPKSCDKTHTCP

SEQ ID NO: 80 - protein, 113 aa, synthetic construct
  source 1..113: note = synthetic polypeptide
PCPAPEAAGGPSVFLFPPKPKDTLMISRTPEVTCVVVDVSHEDPEVKFNWYVDGVEVHNAKTKPREEQYNSTYRVVSVLTVLHQDWLNGKEYKCKVSNKALPAPIEKTISKAK

SEQ ID NO: 81 - protein, 107 aa, synthetic construct
  source 1..107: note = synthetic polypeptide
GQPREPQVYTLPPSRDELTKNQVSLTCLVKGFYPSDIAVEWESNGQPENNYKTTPPVLDSDGSFFLYSKLTVDKSRWQQGNVFSCSVMHEALHNHYTQKSLSLSPGK

SEQ ID NO: 82 - protein, 446 aa, synthetic construct
  source 1..446: note = synthetic polypeptide
EVQLVESGGGLVQPGGSLRLSCAASGFTFSNYGMHWVRQAPGKGLEWVSYISSGSSTIYYADSVKGRFTISRDNAKNSLYLQMNSLRAEDTAVYYCARRGLLLDYWGQGTTVTVSSASTKGPSVFPLAPSSKSTSGGTAALGCLVKDYFPEPVTVSWNSGALTSGVHTFPAVLQSSGLYSLSSVVTVPSSSLGTQTYICNVNHKPSNTKVDKKVEPKSCDKTHTCPPCPAPELLGGPSVFLFPPKPKDTLMISRTPEVTCVVVDVSHEDPEVKFNWYVDGVEVHNAKTKPREEQYDSTYRVVSVLTVLHQDWLNGKEYKCKVSNKALPAPIEKTISKAKGQPREPQVYTLPPSRDELTKNQVSLTCLVKGFYPSDIAVEWESNGQPENNYKTTPPVLDSDGSFFLYSKLTVDKSRWQQGNVFSCSVMHEALHNHYTQKSLSLSPGK

SEQ ID NO: 83 - protein, 113 aa, synthetic construct
  source 1..113: note = synthetic polypeptide
PCPAPELLGGPSVFLFPPKPKDTLMISRTPEVTCVVVDVSHEDPEVKFNWYVDGVEVHNAKTKPREEQYDSTYRVVSVLTVLHQDWLNGKEYKCKVSNKALPAPIEKTISKAK

SEQ ID NO: 84 - protein, 446 aa, synthetic construct
  source 1..446: note = synthetic polypeptide
EVQLVESGGGLVQPGGSLRLSCAASGFTFSNYGMHWVRQAPGKGLEWVSYISSGSSTIYYADSVKGRFTISRDNAKNSLYLQMNSLRAEDTAVYYCARRGLLLDYWGQGTTVTVSSASTKGPSVFPLAPSSKSTSGGTAALGCLVKDYFPEPVTVSWNSGALTSGVHTFPAVLQSSGLYSLSSVVTVPSSSLGTQTYICNVNHKPSNTKVDKKVEPKSCDKTHTCPPCPAPEAAGGPSVFLFPPKPKDTLMISRTPEVTCVVVDVSHEDPEVKFNWYVDGVEVHNAKTKPREEQYDSTYRVVSVLTVLHQDWLNGKEYKCKVSNKALPAPIEKTISKAKGQPREPQVYTLPPSRDELTKNQVSLTCLVKGFYPSDIAVEWESNGQPENNYKTTPPVLDSDGSFFLYSKLTVDKSRWQQGNVFSCSVMHEALHNHYTQKSLSLSPGK

SEQ ID NO: 85 - protein, 113 aa, synthetic construct
  source 1..113: note = synthetic polypeptide
PCPAPEAAGGPSVFLFPPKPKDTLMISRTPEVTCVVVDVSHEDPEVKFNWYVDGVEVHNAKTKPREEQYDSTYRVVSVLTVLHQDWLNGKEYKCKVSNKALPAPIEKTISKAK

SEQ ID NO: 86 - protein, 113 aa, synthetic construct
  source 1..113: note = synthetic polypeptide
PCPAPELLGGPSVFLFPPKPKDTLMISRTPEVTCVVVDVSHEDPEVKFNWYVDGVEVHNAKTKPREEQYNSTYRVVSVLTVLHQDWLNGKEYKCKVSNKALPAPIEKTISKAK

SEQ ID NO: 87 - protein, 218 aa, synthetic construct
  source 1..218: note = synthetic polypeptide
DIQMTQSPSSLSASLGDRATITCRASKTVSTSSYSYMHWYQQKPGQPPKLLIKYASYLESGVPSRFSGSGSGTDFTLTISSLQPEDAATYYCQHSREFPWTFGGGTKLEIKRTVAAPSVFIFPPSDEQLKSGTASVVCLLNNFYPREAKVQWKVDNALQSGNSQESVTEQDSKDSTYSLSSTLTLSKADYEKHKVYACEVTHQGLSSPVTKSFNRGEC

SEQ ID NO: 88 - protein, 31 aa, synthetic construct
  source 1..31: note = synthetic polypeptide
RASKSVSTSSYSYMHWYQQKPGQPPKLLIKY

SEQ ID NO: 89 - protein, 31 aa, synthetic construct
  source 1..31: note = synthetic polypeptide
RASKTVSTSSYSYMHWYQQKPGQPPKLLIKY

SEQ ID NO: 90 - protein, 33 aa, synthetic construct
  source 1..33: note = synthetic polypeptide
RVTITCRASKSVSTSSYSYMHWYQQKPGKAPKL

SEQ ID NO: 91 - protein, 32 aa, synthetic construct
  VARIANT 1: note = X = any amino acid, but preferentially is a basic residue (R or K)
  VARIANT 30: note = X = any amino acid, but preferentially is a basic residue (R or K)
  source 1..32: note = synthetic polypeptide
XRASKTVSTSSYSYMHWYQQKPGQPPKLLXKY

SEQ ID NO: 92 - protein, 115 aa, synthetic construct
  source 1..115: note = synthetic polypeptide
EVQLVESGGGLVKPGGSRKLSCAASGFTFSDYGMHWVRQAPEKGLEWVAYISSGSSTIYYADTVKGRFTISRDNAKNTLFLQMTSLRSEDTAMYYCARRGLLLDYWGQGTTLTVS

SEQ ID NO: 93 - protein, 132 aa, synthetic construct
  source 1..132: note = synthetic polypeptide
DIVLTQSPASLAVSLGQRATISCRASKSVSTSSYSYMHWYQQKPGQPPKLLIKYASYLESGVPARFSGSGSGTDFTLNIHPVEEEDAATYYCQHSREFPWTFGGGTKLEIKRADAAPGGGGSGGGGSGGGGS